European Patent Application EP 4 130 274 A1, published February 8, 2023. Title: Methods for Editing Target RNA. Applicant: EditForce, Inc. NATIONAL UNIVERSITY CORPORATION TOKAI NATIONAL HIGHER EDUCATION AND RESEARCH SYSTEM KYUSHU UNIVERSITY, NATIONAL UNIVERSITY CORPORATION. The sequence listing filed with the application follows.

SEQUENCE LISTING (96 sequences)

SEQ ID NO: 1 - protein, 136 aa, Artificial Sequence
  DYW:PG
EPGCSWIEVNNKVHEFVAGDKSHPQTKEIYAELERLSKQMKEAGYVPDTKFVLHDVEEEEKEQLLCYHSEKLAIAFGLISTPPGTPLRIIKNLRVCGDCHTATKFISKIVGREIVVRDANRFHHFKDGVCSCGDYW

SEQ ID NO: 2 - protein, 137 aa, Artificial Sequence
  DYW:WW
KPGQSWWTDTGGIVHTFVVGDTKHPQSQDIYAKLKDLYVKMKEEGYVPHLDCVLWDISDDEKEDALCGHSEKLAIACALINTPPGTPIRIVKNLRVCDDCHKAIALISKIEGRNIICRDASRFHNYKDGKCSCGDYW

SEQ ID NO: 3 - protein, 133 aa, Artificial Sequence
  DYW:KP
KPASALIEVNKKVHEFVVGNNQSEEISAMLKSLNSRMKEEGHVPNLDLVLKPVSDEEKEAALCEHAEKLAIAFGLLNTPQGQTLRVTKNLRMCNDCHNASKIISKIERREIILRDDCCIHHFKDGLCSCGDMF

SEQ ID NO: 4 - protein, 35 aa, Artificial Sequence
  P1 motif
FSWNSMIRGYARSGQPEEALSLFSQMRRSGIKPDS

SEQ ID NO: 5 - protein, 35 aa, Artificial Sequence
  L1 motif
YTFPFVLKACASLSSLEEGKQIHAHVIKSGFESDV

SEQ ID NO: 6 - protein, 31 aa, Artificial Sequence
  S1 motif
YVQSSLIDMYAKCGSLEDARKVFDEMPERNV

SEQ ID NO: 7 - protein, 35 aa, Artificial Sequence
  P1 motif
VSWNAMISGYAQNGQSEEALELFREMQKEGIKPSE

SEQ ID NO: 8 - protein, 35 aa, Artificial Sequence
  L1 motif
FTFCSVLKACASLGSLEMGKQIHGYVIKSGFESIV

SEQ ID NO: 9 - protein, 31 aa, Artificial Sequence
  S1 motif
FVGNALIDMYAKCGSLEDARKVFDEMPERTV

SEQ ID NO: 10 - protein, 35 aa, Artificial Sequence
  P1 motif
VSWTAMISGYAQNGQSEEALELFREMQREGVKPDE

SEQ ID NO: 11 - protein, 35 aa, Artificial Sequence
  L1 motif
VTLPSVLSACANLGALEQGKQIHAYVIKNGFESDV

SEQ ID NO: 12 - protein, 31 aa, Artificial Sequence
  S1 motif
FVGSALIDMYAKCGSIEEARKVFDEMPEKDV

SEQ ID NO: 13 - protein, 35 aa, Artificial Sequence
  P motif
VTYTTLIDGLCKAGKVDEALELFKEMRSKGVKPNV

SEQ ID NO: 14 - protein, 35 aa, Artificial Sequence
  P motif
VTYNTLIDGLCKAGRLDEAEELLEEMEEKGIKPDV

SEQ ID NO: 15 - protein, 35 aa, Artificial Sequence
  P motif
VTYNTLIDGLCKSGKIEEALKLFKEMEEKGITPSV

SEQ ID NO: 16 - protein, 35 aa, Artificial Sequence
  P motif
VTYTTLIDGLCKAGKVDEALELFDEMKERGIKPDV

SEQ ID NO: 17 - protein, 35 aa, Artificial Sequence
  P2 motif
VSWNAMIAAYAQHGHGKEALQLFQQMQQEGVKPSE

SEQ ID NO: 18 - protein, 36 aa, Artificial Sequence
  L2 motif
VTFTSILSACSHAGLVDEGHHYFESMSPDYGITPRV

SEQ ID NO: 19 - protein, 32 aa, Artificial Sequence
  S2 motif
EHYGCMVDLLGRAGRLDEAEDLIKSMPFQPNV

SEQ ID NO: 20 - protein, 34 aa, Artificial Sequence
  E1 motif
VVWGTLLGACRVHGDVERGERAAERILELDPESA

SEQ ID NO: 21 - protein, 33 aa, Artificial Sequence
  E2 motif
APYVLLSNIYAAAGRWDEAAKVRKLMKERGVKK

SEQ ID NO: 22 - protein, 35 aa, Artificial Sequence
  P2 motif
VTWNALIAGYARQGESDLVFHLLERMRQEGIQPSG

SEQ ID NO: 23 - protein, 36 aa, Artificial Sequence
  L2 motif
VTFTSVLTVCSHAGLVDEGQKYFDAMSEDYGITPRI

SEQ ID NO: 24 - protein, 32 aa, Artificial Sequence
  S2 motif
EHYGCMVDLLGRAGQMDEAVAMVEKMPFQPNL

SEQ ID NO: 25 - protein, 34 aa, Artificial Sequence
  E1 motif
VTWGTLLGACRKWNNVEIGRHAFECAVRLDEKSA

SEQ ID NO: 26 - protein, 33 aa, Artificial Sequence
  E2 motif
AAYVLMSNIYADAHMWEERDKIQAMRKNARAWK

SEQ ID NO: 27 - protein, 35 aa, Artificial Sequence
  P2 motif
VAWNSMIKGYGMNHEGKMAVQCFEDMQKQGVKPSA

SEQ ID NO: 28 - protein, 36 aa, Artificial Sequence
  L2 motif
VTFTCLLTACSHASLVSEGQEYFKMMREEYGIAPRV

SEQ ID NO: 29 - protein, 31 aa, Artificial Sequence
  S2 motif
EHYGCMVDLLARSGHLYEAEKFLEMLCPPNE

SEQ ID NO: 30 - protein, 34 aa, Artificial Sequence
  E1 motif
GTWGALLSACKTYGEVELGLRCFQQLVQLNPESA

SEQ ID NO: 31 - protein, 33 aa, Artificial Sequence
  E2 motif
AWYVLMADIYAGAGRWDDAYRIEELRKHAGAKK

SEQ ID NO: 32 - protein, 7 aa, Simian virus 40
PKKKRKV

SEQ ID NO: 33 - protein, 16 aa, Artificial Sequence
  nucleoplasmin NLS
KRPAATKKAGQAKKKK

SEQ ID NO: 34 - RNA, 17 nt, Artificial Sequence
  Taget sequence
auuacacgugcaaaauy

SEQ ID NO: 35 - protein, 610 aa, Artificial Sequence
  PLS array (3 P1L1S1 triplets) + DYW:PG-lyc
VFSWNSMIRGYARNGQPEEALSLYSQMRRSGIKPDNYTFPFVLKACASLSSLKEGKQIHGHVIKSGFESDVYVQSALIDMYAKCGELEDARKVFDEMPERNVVSWNAMISGYAQNGQSEEALELFREMQQEGIKPSEFTFCSVLSACASLGSLEMGKQIHGYVIKSGFESIVFVGNALIDMYAKCGSIEDARKVFDEMPERTVVSWTAMISGYAQNGQSEEALELFREMQREGVKPDEVTLPSVLSACANLGALEQGKQIHAYVIKSGFESDVFVGSALIDMYAKCGSIEDARKVFDKMPERDVVSWNAMIAAYAQHGHGKEALQLFQQMQQEGVKPSEVTFTSILSACSHAGLVDEGHHYFESMSPDYGITPRVEHYGCMVDLLGRAGRLDEAEDLIKSMPFQPNVVVWGTLLGACRVHGDVERGERAAERILELDPESAAPYVLLSNIYAAAGRWDEAAKVRKLMKERGVKKEPGCSWIEVNNKVHEFVAGDKSHPQTKEIYAELERLSKQMKEAGYVPDTKFVLHDVEEEEKEQLLCYHSEKLAIAFGLISTPPGTPLRIIKNLRVCGDCHTATKFISKIVGREIVVRDANRFHHFKDGVCSCGDYW

SEQ ID NO: 36 - protein, 611 aa, Artificial Sequence
  PLS array (3 P1L1S1 triplets) + DYW:WW-WW5
VFSWNSMIRGYARNGQPEEALSLYSQMRRSGIKPDNYTFPFVLKACASLSSLKEGKQIHGHVIKSGFESDVYVQSALIDMYAKCGELEDARKVFDEMPERNVVSWNAMISGYAQNGQSEEALELFREMQQEGIKPSEFTFCSVLSACASLGSLEMGKQIHGYVIKSGFESIVFVGNALIDMYAKCGSIEDARKVFDEMPERTVVSWTAMISGYAQNGQSEEALELFREMQREGVKPDEVTLPSVLSACANLGALEQGKQIHAYVIKSGFESDVFVGSALIDMYAKCGSIEDARKVFDKMPERDVVTWNALIAGYARQGESDLVFHLLERMRQEGIQPSGVTFTSVLTVCSHAGLVDEGQKYFDAMSEDYGITPRIEHYGCMVDLLGRAGQMDEAVAMVEKMPFQPNLVTWGTLLGACRKWNNVEIGRHAFECAVRLDEKSAAAYVLMSNIYADAHMWEERDKIQAMRKNARAWKKPGQSWWTDTGGIVHTFVVGDTKHPQSQDIYAKLKDLYVKMKEEGYVPHLDCVLWDISDDEKEDALCGHSEKLAIACALINTPPGTPIRIVKNLRVCDDCHKAIALISKIEGRNIICRDASRFHNYKDGKCSCGDYW

SEQ ID NO: 37 - protein, 606 aa, Artificial Sequence
  PLS array (P1L1S1 triplets) + DYW:KP-lepto
VFSWNSMIRGYARNGQPEEALSLYSQMRRSGIKPDNYTFPFVLKACASLSSLKEGKQIHGHVIKSGFESDVYVQSALIDMYAKCGELEDARKVFDEMPERNVVSWNAMISGYAQNGQSEEALELFREMQQEGIKPSEFTFCSVLSACASLGSLEMGKQIHGYVIKSGFESIVFVGNALIDMYAKCGSIEDARKVFDEMPERTVVSWTAMISGYAQNGQSEEALELFREMQREGVKPDEVTLPSVLSACANLGALEQGKQIHAYVIKSGFESDVFVGSALIDMYAKCGSIEDARKVFDKMPERDVVAWNSMIKGYGMNHEGKMAVQCFEDMQKQGVKPSAVTFTCLLTACSHASLVSEGQEYFKMMREEYGIAPRVEHYGCMVDLLARSGHLYEAEKFLEMLCPPNEGTWGALLSACKTYGEVELGLRCFQQLVQLNPESAAWYVLMADIYAGAGRWDDAYRIEELRKHAGAKKKPASALIEVNKKVHEFVVGNNQSEEISAMLKSLNSRMKEEGHVPNLDLVLKPVSDEEKEAALCEHAEKLAIAFGLLNTPQGQTLRVTKNLRMCNDCHNASKIISKIERREIILRDDCCIHHFKDGLCSCGDMF

SEQ ID NO: 38 - protein, 657 aa, Artificial Sequence
  P array (10 PPR motifs) + DYW:PG-lyc
VVTYTTLIDGLCKAGKVDEALELFKEMRSKGVKPNVVTYNTLIDGLCKAGRLDEAEELLEEMEEKGIKPDVVTYNTLIDGLCKAGRLDEAEELLEEMEEKGIKPDVVTYTTLIDGLCKAGKVDEALELFKEMRSKGVKPNVVTYNTLIDGLCKSGKIEEALKLFKEMEEKGITPSVVTYTTLIDGLCKAGKVDEALELFKEMRSKGVKPNVVTYNTLIDGLCKSGKIEEALKLFKEMEEKGITPSVVTYTTLIDGLCKAGKVDEALELFDEMKERGIKPDVVTYNTLIDGLCKAGRLDEAEELLEEMEEKGIKPDVVTYTTLIDGLCKAGKVDEALELFDEMKERGIKPDVVSWNAMIAAYAQHGHGKEALQLFQQMQQEGVKPSEVTFTSILSACSHAGLVDEGHHYFESMSPDYGITPRVEHYGCMVDLLGRAGRLDEAEDLIKSMPFQPNVVVWGTLLGACRVHGDVERGERAAERILELDPESAAPYVLLSNIYAAAGRWDEAAKVRKLMKERGVKKEPGCSWIEVNNKVHEFVAGDKSHPQTKEIYAELERLSKQMKEAGYVPDTKFVLHDVEEEEKEQLLCYHSEKLAIAFGLISTPPGTPLRIIKNLRVCGDCHTATKFISKIVGREIVVRDANRFHHFKDGVCSCGDYW

SEQ ID NO: 39 - protein, 658 aa, Artificial Sequence
  P array (10 PPR motifs) + DYW:WW-WW5
VVTYTTLIDGLCKAGKVDEALELFKEMRSKGVKPNVVTYNTLIDGLCKAGRLDEAEELLEEMEEKGIKPDVVTYNTLIDGLCKAGRLDEAEELLEEMEEKGIKPDVVTYTTLIDGLCKAGKVDEALELFKEMRSKGVKPNVVTYNTLIDGLCKSGKIEEALKLFKEMEEKGITPSVVTYTTLIDGLCKAGKVDEALELFKEMRSKGVKPNVVTYNTLIDGLCKSGKIEEALKLFKEMEEKGITPSVVTYTTLIDGLCKAGKVDEALELFDEMKERGIKPDVVTYNTLIDGLCKAGRLDEAEELLEEMEEKGIKPDVVTYTTLIDGLCKAGKVDEALELFDEMKERGIKPDVVTWNALIAGYARQGESDLVFHLLERMRQEGIQPSGVTFTSVLTVCSHAGLVDEGQKYFDAMSEDYGITPRIEHYGCMVDLLGRAGQMDEAVAMVEKMPFQPNLVTWGTLLGACRKWNNVEIGRHAFECAVRLDEKSAAAYVLMSNIYADAHMWEERDKIQAMRKNARAWKKPGQSWWTDTGGIVHTFVVGDTKHPQSQDIYAKLKDLYVKMKEEGYVPHLDCVLWDISDDEKEDALCGHSEKLAIACALINTPPGTPIRIVKNLRVCDDCHKAIALISKIEGRNIICRDASRFHNYKDGKCSCGDYW

SEQ ID NO: 40 - protein, 653 aa, Artificial Sequence
  P array (10 PPR motifs) + DYW:KP-lepto
VVTYTTLIDGLCKAGKVDEALELFKEMRSKGVKPNVVTYNTLIDGLCKAGRLDEAEELLEEMEEKGIKPDVVTYNTLIDGLCKAGRLDEAEELLEEMEEKGIKPDVVTYTTLIDGLCKAGKVDEALELFKEMRSKGVKPNVVTYNTLIDGLCKSGKIEEALKLFKEMEEKGITPSVVTYTTLIDGLCKAGKVDEALELFKEMRSKGVKPNVVTYNTLIDGLCKSGKIEEALKLFKEMEEKGITPSVVTYTTLIDGLCKAGKVDEALELFDEMKERGIKPDVVTYNTLIDGLCKAGRLDEAEELLEEMEEKGIKPDVVTYTTLIDGLCKAGKVDEALELFDEMKERGIKPDVVAWNSMIKGYGMNHEGKMAVQCFEDMQKQGVKPSAVTFTCLLTACSHASLVSEGQEYFKMMREEYGIAPRVEHYGCMVDLLARSGHLYEAEKFLEMLCPPNEGTWGALLSACKTYGEVELGLRCFQQLVQLNPESAAWYVLMADIYAGAGRWDDAYRIEELRKHAGAKKKPASALIEVNKKVHEFVVGNNQSEEISAMLKSLNSRMKEEGHVPNLDLVLKPVSDEEKEAALCEHAEKLAIAFGLLNTPQGQTLRVTKNLRMCNDCHNASKIISKIERREIILRDDCCIHHFKDGLCSCGDMF

SEQ ID NO: 41 - protein, 136 aa, Artificial Sequence
  PG2
QPGCSSIEVDNKVHEFIVGDRSHPQTEEIYAELERLNKQMKEAGYVPDTRLVLHDVDEEEKEHLLCHHSEKLAIAFGLISTPPGTPLRIIKNLRVCGDCHTATKYISKIVGREIIVRDANRFHHFKDGVCSCGDYW

SEQ ID NO: 42 - protein, 136 aa, Artificial Sequence
  PG3
KPGCSWIEVNNKVHEFVAGDKSHPQTKEIYAELERLSKQMKEAGYVPDTKFVLHDVEEEEKEQLLCYHSEKLAIAFGLISTPPGTPLRIIKNLRVCGDCHTATKFISKIVGREIVVRDANRFHHFKDGVCSCGDYW

SEQ ID NO: 43 - protein, 136 aa, Artificial Sequence
  PG4
EPACSWIEVNNKVHEFVAGDKSHPQTKEIYAELERLSKQMKEAGYVPDTKFVLHDVEEEEKEQLLCYHSEKLAIAFGLISTPPGTPLRIIKNLRVCGDCHTATKFISKIVGREIVVRDANRFHHFKDGVCSCGDYW

SEQ ID NO: 44 - protein, 136 aa, Artificial Sequence
  PG5
EPGCAWIEVNNKVHEFVAGDKSHPQTKEIYAELERLSKQMKEAGYVPDTKFVLHDVEEEEKEQLLCYHSEKLAIAFGLISTPPGTPLRIIKNLRVCGDCHTATKFISKIVGREIVVRDANRFHHFKDGVCSCGDYW

SEQ ID NO: 45 - protein, 136 aa, Artificial Sequence
  PG6
EPGCSTIEVNNKVHEFVAGDKSHPQTKEIYAELERLSKQMKEAGYVPDTKFVLHDVEEEEKEQLLCYHSEKLAIAFGLISTPPGTPLRIIKNLRVCGDCHTATKFISKIVGREIVVRDANRFHHFKDGVCSCGDYW

SEQ ID NO: 46 - protein, 136 aa, Artificial Sequence
  PG7
EPGCSWIEVNNKVHEFVAGDKSHPQTKEIYAELERLNKQMKEAGYVPDTKFVLHDVEEEEKEQLLCYHSEKLAIAFGLISTPPGTPLRIIKNLRVCGDCHTATKFISKIVGREIVVRDANRFHHFKDGVCSCGDYW

SEQ ID NO: 47 - protein, 136 aa, Artificial Sequence
  PG8
EPGCSWIEVNNKVHEFVAGDKSHPQTKEIYAELERLSKQMKEAGHVPDTKFVLHDVEEEEKEQLLCYHSEKLAIAFGLISTPPGTPLRIIKNLRVCGDCHTATKFISKIVGREIVVRDANRFHHFKDGVCSCGDYW

SEQ ID NO: 48 - protein, 136 aa, Artificial Sequence
  PG9
EPGCSWIEVNNKVHEFVAGDKSHPQTKEIYAELERLSKQMKEAGYVPDTKFVLHPVEEEEKEQLLCYHSEKLAIAFGLISTPPGTPLRIIKNLRVCGDCHTATKFISKIVGREIVVRDANRFHHFKDGVCSCGDYW

SEQ ID NO: 49 - protein, 136 aa, Artificial Sequence
  PG10
EPGCSWIEVNNKVHEFVAGDKSHPQTKEIYAELERLSKQMKEAGYVPDTKFVLHDVEEEEKEQLLCYHSEKLAIAFGLISTPPGTPLRVTKNLRVCGDCHTATKFISKIVGREIVVRDANRFHHFKDGVCSCGDYW

SEQ ID NO: 50 - protein, 136 aa, Artificial Sequence
  PG11
EPGCSWIEVNNKVHEFVAGDKSHPQTKEIYAELERLSKQMKEAGYVPDTKFVLHDVEEEEKEQLLCYHSEKLAIAFGLISTPPGTPLRIIKNLRMCGDCHTATKFISKIVGREIVVRDANRFHHFKDGVCSCGDYW

SEQ ID NO: 51 - protein, 136 aa, Artificial Sequence
  PG12
EPGCSWIEVNNKVHEFVAGDKSHPQTKEIYAELERLSKQMKEAGYVPDTKFVLHDVEEEEKEQLLCYHSEKLAIAFGLISTPPGTPLRIIKNLRVCGDCHTATKFISKIVKREIVVRDANRFHHFKDGVCSCGDYW

SEQ ID NO: 52 - protein, 136 aa, Artificial Sequence
  PG13
EPGCSWIEVNNKVHEFVAGDKSHPQTKEIYAELERLSKQMKEAGYVPDTKFVLHDVEEEEKEQLLCYHSEKLAIAFGLISTPPGTPLRIIKNLRVCGDCHTATKFISKIVGREIVVRDDCRFHHFKDGVCSCGDYW

SEQ ID NO: 53 - protein, 136 aa, Artificial Sequence
  PG14
EPGCSWIEVNNKVHEFVAGDKSHPQTKEIYAELERLSKQMKEAGYVPDTKFVLHDVEEEEKEQLLCYHSEKLAIAFGLISTPPGTPLRIIKNLRVCGDCHTATKFISKIVGREIVVRDANCVHHFKDGVCSCGDYW

SEQ ID NO: 54 - protein, 137 aa, Artificial Sequence
  WW2
QPGQSWWTDMGGVVHTFVVGDREHPESQDIYAKLKDLIVKMKKEGYVPHLDSVLRDIPDDEKEDALCGHSEKLAIAYALLKTPEGTTIRVVKNLRVCEDCHTATALISKIEQRTIICRDASRFHVYKDGKCSCGDYW

SEQ ID NO: 55 - protein, 137 aa, Artificial Sequence
  WW3
EPGQSWWTDTGGIVHTFVVGDTKHPQSQDIYAKLKDLYVKMKEEGYVPHLDCVLWDISDDEKEDALCGHSEKLAIACALINTPPGTPIRIVKNLRVCDDCHKAIALISKIEGRNIICRDASRFHNYKDGKCSCGDYW

SEQ ID NO: 56 - protein, 137 aa, Artificial Sequence
  WW4
KPAQSWWTDTGGIVHTFVVGDTKHPQSQDIYAKLKDLYVKMKEEGYVPHLDCVLWDISDDEKEDALCGHSEKLAIACALINTPPGTPIRIVKNLRVCDDCHKAIALISKIEGRNIICRDASRFHNYKDGKCSCGDYW

SEQ ID NO: 57 - protein, 137 aa, Artificial Sequence
  WW5
KPGQAWWTDTGGIVHTFVVGDTKHPQSQDIYAKLKDLYVKMKEEGYVPHLDCVLWDISDDEKEDALCGHSEKLAIACALINTPPGTPIRIVKNLRVCDDCHKAIALISKIEGRNIICRDASRFHNYKDGKCSCGDYW

SEQ ID NO: 58 - protein, 137 aa, Artificial Sequence
  WW6
KPGQSTWTDTGGIVHTFVVGDTKHPQSQDIYAKLKDLYVKMKEEGYVPHLDCVLWDISDDEKEDALCGHSEKLAIACALINTPPGTPIRIVKNLRVCDDCHKAIALISKIEGRNIICRDASRFHNYKDGKCSCGDYW

SEQ ID NO: 59 - protein, 136 aa, Artificial Sequence
  WW7
KPGQSWTDTGGIVHTFVVGDTKHPQSQDIYAKLKDLYVKMKEEGYVPHLDCVLWDISDDEKEDALCGHSEKLAIACALINTPPGTPIRIVKNLRVCDDCHKAIALISKIEGRNIICRDASRFHNYKDGKCSCGDYW

SEQ ID NO: 60 - protein, 137 aa, Artificial Sequence
  WW8
KPGQSWWTDTGGIVHTFVVGDTKHPQSQDIYAKLKDLNVKMKEEGYVPHLDCVLWDISDDEKEDALCGHSEKLAIACALINTPPGTPIRIVKNLRVCDDCHKAIALISKIEGRNIICRDASRFHNYKDGKCSCGDYW

SEQ ID NO: 61 - protein, 137 aa, Artificial Sequence
  WW9
KPGQSWWTDTGGIVHTFVVGDTKHPQSQDIYAKLKDLYVKMKEEGHVPHLDCVLWDISDDEKEDALCGHSEKLAIACALINTPPGTPIRIVKNLRVCDDCHKAIALISKIEGRNIICRDASRFHNYKDGKCSCGDYW

SEQ ID NO: 62 - protein, 137 aa, Artificial Sequence
  WW10
KPGQSWWTDTGGIVHTFVVGDTKHPQSQDIYAKLKDLYVKMKEEGYVPHLDCVLWPISDDEKEDALCGHSEKLAIACALINTPPGTPIRIVKNLRVCDDCHKAIALISKIEGRNIICRDASRFHNYKDGKCSCGDYW

SEQ ID NO: 63 - protein, 137 aa, Artificial Sequence
  WW11
KPGQSWWTDTGGIVHTFVVGDTKHPQSQDIYAKLKDLYVKMKEEGYVPHLDCVLWDISDDEKEDALCGHSEKLAIACALINTPPGTPIRVTKNLRVCDDCHKAIALISKIEGRNIICRDASRFHNYKDGKCSCGDYW

SEQ ID NO: 64 - protein, 137 aa, Artificial Sequence
  WW12
KPGQSWWTDTGGIVHTFVVGDTKHPQSQDIYAKLKDLYVKMKEEGYVPHLDCVLWDISDDEKEDALCGHSEKLAIACALINTPPGTPIRIVKNLRMCDDCHKAIALISKIEGRNIICRDASRFHNYKDGKCSCGDYW

SEQ ID NO: 65 - protein, 137 aa, Artificial Sequence
  WW13
KPGQSWWTDTGGIVHTFVVGDTKHPQSQDIYAKLKDLYVKMKEEGYVPHLDCVLWDISDDEKEDALCGHSEKLAIACALINTPPGTPIRIVKNLRVCDDCHKAIALISKIEKRNIICRDASRFHNYKDGKCSCGDYW

SEQ ID NO: 66 - protein, 137 aa, Artificial Sequence
  WW14
KPGQSWWTDTGGIVHTFVVGDTKHPQSQDIYAKLKDLYVKMKEEGYVPHLDCVLWDISDDEKEDALCGHSEKLAIACALINTPPGTPIRIVKNLRVCDDCHKAIALISKIEGRNIICRDDCRFHNYKDGKCSCGDYW

SEQ ID NO: 67 - protein, 137 aa, Artificial Sequence
  WW15
KPGQSWWTDTGGIVHTFVVGDTKHPQSQDIYAKLKDLYVKMKEEGYVPHLDCVLWDISDDEKEDALCGHSEKLAIACALINTPPGTPIRIVKNLRVCDDCHKAIALISKIEGRNIICRDASCVHNYKDGKCSCGDYW

SEQ ID NO: 68 - protein, 133 aa, Artificial Sequence
  KP2
KPAVAGIEVDRHVHTFVVGEERGDISCKVRSMNTRLKEEGGHVPHTELVLKPLSEKEKEDELCGHAEKLALAYGLLNTPDGTPLLVTKNLRMCRDCHSSTEIMSRIEKREIVVRDAHRVHRFVDGSCSCGGRP

SEQ ID NO: 69 - protein, 133 aa, Artificial Sequence
  KP3
KPAVATIEVNKQVHRFLVGERREDIALKVESTNARLKQEGGHVPHTKLVLKPLCEKEKEDALCGHAEKLALAFGLLNTPSGTPLVVTKNLRMCSDCHSSTEIMSRLEQRDIVVRDGYRVHRFAAGCCSCKGRP

SEQ ID NO: 70 - protein, 133 aa, Artificial Sequence
  KP4
KPAVATIEVNKQVHRFLVGERREDIALKVESTNARLKQEGGHVPHTKLVLKPLCEKEKEDVLCGHAEKLALAFGLLNTPSGTPLVVTKNLRMCSDCHSSTEIMSRLEQRDIVVRDGYRVHRFANGCCSCKGRP

SEQ ID NO: 71 - protein, 133 aa, Artificial Sequence
  KP5
KPGSALIEVNKKVHEFVVGNNQSEEISAMLKSLNSRMKEEGHVPNLDLVLKPVSDEEKEAALCEHAEKLAIAFGLLNTPQGQTLRVTKNLRMCNDCHNASKIISKIERREIILRDDCCIHHFKDGLCSCGDMF

SEQ ID NO: 72 - protein, 137 aa, Artificial Sequence
  KP6
KPAQSWWTDTGGIVHTFVVGDTKHPQSEEISAMLKSLNSRMKEEGHVPNLDLVLKPVSDEEKEAALCEHAEKLAIAFGLLNTPQGQTLRVTKNLRMCNDCHNASKIISKIERREIILRDDCCIHHFKDGLCSCGDYW

SEQ ID NO: 73 - protein, 133 aa, Artificial Sequence
  KP7
KPASSLIEVNKKVHEFVVGNNQSEEISAMLKSLNSRMKEEGHVPNLDLVLKPVSDEEKEAALCEHAEKLAIAFGLLNTPQGQTLRVTKNLRMCNDCHNASKIISKIERREIILRDDCCIHHFKDGLCSCGDMF

SEQ ID NO: 74 - protein, 137 aa, Artificial Sequence
  KP8
KPGQAWWTDTGGIVHTFVVGDTKHPQSEEISAMLKSLNSRMKEEGHVPNLDLVLKPVSDEEKEAALCEHAEKLAIAFGLLNTPQGQTLRVTKNLRMCNDCHNASKIISKIERREIILRDDCCIHHFKDGLCSCGDYW

SEQ ID NO: 75 - protein, 133 aa, Artificial Sequence
  KP9
KPASAWIEVNKKVHEFVVGNNQSEEISAMLKSLNSRMKEEGHVPNLDLVLKPVSDEEKEAALCEHAEKLAIAFGLLNTPQGQTLRVTKNLRMCNDCHNASKIISKIERREIILRDDCCIHHFKDGLCSCGDMF

SEQ ID NO: 76 - protein, 137 aa, Artificial Sequence
  KP10
KPGQSTWTDTGGIVHTFVVGDTKHPQSEEISAMLKSLNSRMKEEGHVPNLDLVLKPVSDEEKEAALCEHAEKLAIAFGLLNTPQGQTLRVTKNLRMCNDCHNASKIISKIERREIILRDDCCIHHFKDGLCSCGDYW

SEQ ID NO: 77 - protein, 136 aa, Artificial Sequence
  KP11
KPGQSWTDTGGIVHTFVVGDTKHPQSEEISAMLKSLNSRMKEEGHVPNLDLVLKPVSDEEKEAALCEHAEKLAIAFGLLNTPQGQTLRVTKNLRMCNDCHNASKIISKIERREIILRDDCCIHHFKDGLCSCGDYW

SEQ ID NO: 78 - protein, 137 aa, Artificial Sequence
  KP12
KPGQSWWTDTGGIVHTFVVGDTKHPQSEEISAMLKSLSSRMKEEGHVPNLDLVLKPVSDEEKEAALCEHAEKLAIAFGLLNTPQGQTLRVTKNLRMCNDCHNASKIISKIERREIILRDDCCIHHFKDGLCSCGDYW

SEQ ID NO: 79 - protein, 133 aa, Artificial Sequence
  KP13
KPASALIEVNKKVHEFVVGNNQSEEISAMLKSLNSRMKEEGYVPNLDLVLKPVSDEEKEAALCEHAEKLAIAFGLLNTPQGQTLRVTKNLRMCNDCHNASKIISKIERREIILRDDCCIHHFKDGLCSCGDMF

SEQ ID NO: 80 - protein, 137 aa, Artificial Sequence
  KP14
KPGQSWWTDTGGIVHTFVVGDTKHPQSEEISAMLKSLNSRMKEEGYVPNLDLVLKPVSDEEKEAALCEHAEKLAIAFGLLNTPQGQTLRVTKNLRMCNDCHNASKIISKIERREIILRDDCCIHHFKDGLCSCGDYW

SEQ ID NO: 81 - protein, 137 aa, Artificial Sequence
  KP15
KPGQSWWTDTGGIVHTFVVGDTKHPQSEEISAMLKSLNSRMKEEGHVPNLDLVLKDVSDEEKEAALCEHAEKLAIAFGLLNTPQGQTLRVTKNLRMCNDCHNASKIISKIERREIILRDDCCIHHFKDGLCSCGDYW

SEQ ID NO: 82 - protein, 137 aa, Artificial Sequence
  KP16
KPGQSWWTDTGGIVHTFVVGDTKHPQSEEISAMLKSLNSRMKEEGHVPNLDLVLKPVSDEEKEAALCEHAEKLAIAFGLLNTPQGQTLRIVKNLRMCNDCHNASKIISKIERREIILRDDCCIHHFKDGLCSCGDYW

SEQ ID NO: 83 - protein, 133 aa, Artificial Sequence
  KP17
KPASALIEVNKKVHEFVVGNNQSEEISAMLKSLNSRMKEEGHVPNLDLVLKPVSDEEKEAALCEHAEKLAIAFGLLNTPQGQTLRVTKNLRMCNDCHNASKIISKIEGREIILRDDCCIHHFKDGLCSCGDMF

SEQ ID NO: 84 - protein, 137 aa, Artificial Sequence
  KP18
KPGQSWWTDTGGIVHTFVVGDTKHPQSEEISAMLKSLNSRMKEEGHVPNLDLVLKPVSDEEKEAALCEHAEKLAIAFGLLNTPQGQTLRVTKNLRMCNDCHNASKIISKIEGREIILRDDCCIHHFKDGLCSCGDYW

SEQ ID NO: 85 - protein, 133 aa, Artificial Sequence
  KP19
KPASALIEVNKKVHEFVVGNNQSEEISAMLKSLNSRMKEEGHVPNLDLVLKPVSDEEKEAALCEHAEKLAIAFGLLNTPQGQTLRVTKNLRMCNDCHNASKIISKIERREIILRDASCIHHFKDGLCSCGDMF

SEQ ID NO: 86 - protein, 137 aa, Artificial Sequence
  KP20
KPGQSWWTDTGGIVHTFVVGDTKHPQSEEISAMLKSLNSRMKEEGHVPNLDLVLKPVSDEEKEAALCEHAEKLAIAFGLLNTPQGQTLRVTKNLRMCNDCHNASKIISKIERREIILRDASCIHHFKDGLCSCGDYW

SEQ ID NO: 87 - protein, 137 aa, Artificial Sequence
  KP21
KPGQSWWTDTGGIVHTFVVGDTKHPQSEEISAMLKSLNSRMKEEGHVPNLDLVLKPVSDEEKEAALCEHAEKLAIAFGLLNTPQGQTLRVTKNLRMCNDCHNASKIISKIERREIILRDDCCIHHFKDGLCSCGDMF

SEQ ID NO: 88 - protein, 137 aa, Artificial Sequence
  KP22
KPGQSWWTDTGGIVHTFVVGDTKHPQSQDIYAKLKSLNSRMKEEGHVPNLDLVLKPVSDEEKEAALCEHAEKLAIAFGLLNTPQGQTLRVTKNLRMCNDCHNASKIISKIERREIILRDDCCIHHFKDGLCSCGDMF

SEQ ID NO: 89 - protein, 137 aa, Artificial Sequence
  KP23
KPGQSWWTDTGGIVHTFVVGDTKHPQSQDIYAKLKSLNSRMKEEGHVPNLDLVLKPVSDEEKEAALCEHAEKLAIAFGLLNTPQGQTLRVTKNLRMCNDCHNASKIISKIERREIILRDDCCIHHFKDGLCSCGDYW

SEQ ID NO: 90 - protein, 137 aa, Artificial Sequence
  Chimeric KP1a
KPGQSWWTDTGGIVHTFVVGDTKHPQSEEISAMLKSLNSRMKEEGHVPNLDLVLKPVSDEEKEAALCEHAEKLAIAFGLLNTPQGQTLRVTKNLRMCNDCHNASKIISKIERREIILRDDCCIHHFKDGLCSCGDYW

SEQ ID NO: 91 - RNA, 22 nt, Artificial Sequence
  ND2
cccagcuacgcaaaaucuuagc

SEQ ID NO: 92 - RNA, 22 nt, Artificial Sequence
  ND5
augacaucaaaaaaaucguagc

SEQ ID NO: 93 - protein, 830 aa, Artificial Sequence
  MTS-P-PG1_ND2
MALLRAAVSELRRRGRGALTPLPALSSLLSSLSPRSPASTRPEPNNPHADRRHVIALRRCPPLPASAVLAPELLHARGLLPRHWSHASPLSTSSSSSRPADKAQLTWVDKWIPEAARPYSHGSGGSGGGLHMGSGGLSSGDYKDHDGDYKDHDIDYKDDDDKGSGGSGGSGNSVVTYNTLIDGLCKSGKIEEALKLFKEMEEKGITPSVVTYNTLIDGLCKSGKIEEALKLFKEMEEKGITPSVVTYNTLIDGLCKSGKIEEALKLFKEMEEKGITPSVVTYTTLIDGLCKAGKVDEALELFKEMRSKGVKPNVVTYTTLIDGLCKAGKVDEALELFDEMKERGIKPDVVTYNTLIDGLCKSGKIEEALKLFKEMEEKGITPSVVTYNTLIDGLCKAGRLDEAEELLEEMEEKGIKPDVVTYTTLIDGLCKAGKVDEALELFKEMRSKGVKPNVVTYNTLIDGLCKSGKIEEALKLFKEMEEKGITPSVVTYTTLIDGLCKAGKVDEALELFDEMKERGIKPDVVSWNAMIAAYAQHGHGKEALQLFQQMQQEGVKPSEVTFTSILSACSHAGLVDEGHHYFESMSPDYGITPRVEHYGCMVDLLGRAGRLDEAEDLIKSMPFQPNVVVWGTLLGACRVHGDVERGERAAERILELDPESAAPYVLLSNIYAAAGRWDEAAKVRKLMKERGVKKEPGCSWIEVNNKVHEFVAGDKSHPQTKEIYAELERLSKQMKEAGYVPDTKFVLHDVEEEEKEQLLCYHSEKLAIAFGLISTPPGTPLRIIKNLRVCGDCHTATKFISKIVGREIVVRDANRFHHFKDGVCSCGDYW

SEQ ID NO: 94 - protein, 831 aa, Artificial Sequence
  MTS-P-WW1_ND2
MALLRAAVSELRRRGRGALTPLPALSSLLSSLSPRSPASTRPEPNNPHADRRHVIALRRCPPLPASAVLAPELLHARGLLPRHWSHASPLSTSSSSSRPADKAQLTWVDKWIPEAARPYSHGSGGSGGGLHMGSGGLSSGDYKDHDGDYKDHDIDYKDDDDKGSGGSGGSGNSVVTYNTLIDGLCKSGKIEEALKLFKEMEEKGITPSVVTYNTLIDGLCKSGKIEEALKLFKEMEEKGITPSVVTYNTLIDGLCKSGKIEEALKLFKEMEEKGITPSVVTYTTLIDGLCKAGKVDEALELFKEMRSKGVKPNVVTYTTLIDGLCKAGKVDEALELFDEMKERGIKPDVVTYNTLIDGLCKSGKIEEALKLFKEMEEKGITPSVVTYNTLIDGLCKAGRLDEAEELLEEMEEKGIKPDVVTYTTLIDGLCKAGKVDEALELFKEMRSKGVKPNVVTYNTLIDGLCKSGKIEEALKLFKEMEEKGITPSVVTYTTLIDGLCKAGKVDEALELFDEMKERGIKPDVVTWNALIAGYARQGESDLVFHLLERMRQEGIQPSGVTFTSVLTVCSHAGLVDEGQKYFDAMSEDYGITPRIEHYGCMVDLLGRAGQMDEAVAMVEKMPFQPNLVTWGTLLGACRKWNNVEIGRHAFECAVRLDEKSAAAYVLMSNIYADAHMWEERDKIQAMRKNARAWKKPGQSWWTDTGGIVHTFVVGDTKHPQSQDIYAKLKDLYVKMKEEGYVPHLDCVLWDISDDEKEDALCGHSEKLAIACALINTPPGTPIRIVKNLRVCDDCHKAIALISKIEGRNIICRDASRFHNYKDGKCSCGDYW

SEQ ID NO: 95 - protein, 830 aa, Artificial Sequence
  MTS-P-PG1_ND5
MALLRAAVSELRRRGRGALTPLPALSSLLSSLSPRSPASTRPEPNNPHADRRHVIALRRCPPLPASAVLAPELLHARGLLPRHWSHASPLSTSSSSSRPADKAQLTWVDKWIPEAARPYSHGSGGSGGGLHMGSGGLSSGDYKDHDGDYKDHDIDYKDDDDKGSGGSGGSGNSVVTYTTLIDGLCKAGKVDEALELFKEMRSKGVKPNVVTYNTLIDGLCKAGRLDEAEELLEEMEEKGIKPDVVTYTTLIDGLCKAGKVDEALELFDEMKERGIKPDVVTYTTLIDGLCKAGKVDEALELFKEMRSKGVKPNVVTYNTLIDGLCKSGKIEEALKLFKEMEEKGITPSVVTYTTLIDGLCKAGKVDEALELFKEMRSKGVKPNVVTYNTLIDGLCKAGRLDEAEELLEEMEEKGIKPDVVTYNTLIDGLCKSGKIEEALKLFKEMEEKGITPSVVTYTTLIDGLCKAGKVDEALELFKEMRSKGVKPNVVTYTTLIDGLCKAGKVDEALELFKEMRSKGVKPNVVSWTAMIAAYAQHGHGKEALQLFQQMQQEGVKPNEVTFTSILSACSHAGLVDEGHHYFESMSPDYGITPRVEHYGCMVDLLGRAGRLDEAEDLIKSMPFQPNVVVWGTLLGACRVHGDVERGERAAERILELDPESAAPYVLLSNIYAAAGRWDEAAKVRKLMKERGVKKEPGCSWIEVNNKVHEFVAGDKSHPQTKEIYAELERLSKQMKEAGYVPDTKFVLHDVEEEEKEQLLCYHSEKLAIAFGLISTPPGTPLRIIKNLRVCGDCHTATKFISKIVGREIVVRDANRFHHFKDGVCSCGDYW

SEQ ID NO: 96 - protein, 831 aa, Artificial Sequence
  MTS-P-WW1_ND5
MALLRAAVSELRRRGRGALTPLPALSSLLSSLSPRSPASTRPEPNNPHADRRHVIALRRCPPLPASAVLAPELLHARGLLPRHWSHASPLSTSSSSSRPADKAQLTWVDKWIPEAARPYSHGSGGSGGGLHMGSGGLSSGDYKDHDGDYKDHDIDYKDDDDKGSGGSGGSGNSVVTYTTLIDGLCKAGKVDEALELFKEMRSKGVKPNVVTYNTLIDGLCKAGRLDEAEELLEEMEEKGIKPDVVTYTTLIDGLCKAGKVDEALELFDEMKERGIKPDVVTYTTLIDGLCKAGKVDEALELFKEMRSKGVKPNVVTYNTLIDGLCKSGKIEEALKLFKEMEEKGITPSVVTYTTLIDGLCKAGKVDEALELFKEMRSKGVKPNVVTYNTLIDGLCKAGRLDEAEELLEEMEEKGIKPDVVTYNTLIDGLCKSGKIEEALKLFKEMEEKGITPSVVTYTTLIDGLCKAGKVDEALELFKEMRSKGVKPNVVTYTTLIDGLCKAGKVDEALELFKEMRSKGVKPNVVTWTALIAGYARQGESDLVFHLLERMRQEGIQPNGVTFTSVLTVCSHAGLVDEGQKYFDAMSEDYGITPRIEHYGCMVDLLGRAGQMDEAVAMVEKMPFQPNLVTWGTLLGACRKWNNVEIGRHAFECAVRLDEKSAAAYVLMSNIYADAHMWEERDKIQAMRKNARAWKKPGQSWWTDTGGIVHTFVVGDTKHPQSQDIYAKLKDLYVKMKEEGYVPHLDCVLWDISDDEKEDALCGHSEKLAIACALINTPPGTPIRIVKNLRVCDDCHKAIALISKIEGRNIICRDASRFHNYKDGKCSCGDYW